European Patent Specification EP 3 823 992 B1, published December 13, 2023. Title: ANTI-LYPD3 CAR T-CELL THERAPY FOR THE TREATMENT OF CANCER. Applicant: DUKE UNIVERSITY LI, Qi-Jing WANG, Xiao-Fan CHONG, Mengyang CHEN, Rui. The sequence listing filed with the application follows.

SEQUENCE LISTING (20 sequences)

SEQ ID NO: 1 - DNA, 800 bp, Artificial Sequence
  Synthetic
atggctctgcccgtcaccgccctgctgctgcctctggctctgctgctgcacgccgcacgacccgaagtccagctgctggaaagtgggggaggcctggtgcagccaggaggctctctgaggctgagctgcgcagcatccggcttcacctttagcaacgcatggatgtcctgggtgaggcaggcacctggcaagggcctggagtgggtgtcctacatcagctcctctggctctacaatctactatgccgacagcgtgaagggcaggttcaccatctctagagataacagcaagaatacactgtatctgcagatgaattccctgagggccgaggacaccgccgtgtactattgcgccagagagggcctgtgggcctttgataagtggggccagggcaccctggtgacagtgagctccggaggaggaggatctggcggaggaggcagcggcggcggcggctctcagagcgtgctgacccagccaccttccgcctctggaacaccaggccagagagtgaccatctcctgtacaggctctagctccaacatcggcgccggctacgtggtgcactggtatcagcagctgccaggaaccgcaccaaagctgctgatctacgacaacaataagcggcctagcggcgtgccagatcgcttcagcggctccaagtctggcacaagcgcctccctggcaatctccggcctgcggtctgaggacgaggcagattactattgtgccgcctttgacgatcgcctgaatggacccgtgttcggaggagggactaaactgaccgtgctgggacaggc

SEQ ID NO: 2 - DNA, 249 bp, Artificial Sequence
  Synthetic
ttcgtgccggtcttcctgccagcgaagcccaccacgacgccagcgccgcgaccaccaacaccggcgcccaccatcgcgtcgcagcccctgtccctgcgcccagaggcgtgccggccagcggcggggggcgcagtgcacacgagggggctggacttcgcctgtgatatctacatctgggcgcccttggccgggacttgtggggtccttctcctgtcactggttatcaccctttactgcaaccacaggaac

SEQ ID NO: 3 - DNA, 123 bp, Artificial Sequence
  Synthetic
aggagtaagaggagcaggctcctgcacagtgactacatgaacatgactccccgccgccccgggcccacccgcaagcattaccagccctatgccccaccacgcgacttcgcagcctatcgctcc

SEQ ID NO: 4 - DNA, 141 bp, Artificial Sequence
  Synthetic
cgtttctctgttgttaaacggggcagaaagaagctcctgtatatattcaaacaaccatttatgagaccagtacaaactactcaagaggaagatggctgtagctgccgatttccagaagaagaagaaggaggatgtgaactg

SEQ ID NO: 5 - DNA, 339 bp, Artificial Sequence
  Synthetic
agagtgaagttcagcaggagcgcagacgcccccgcgtaccagcagggccagaaccagctctataacgagctcaatctaggacgaagagaggagtacgatgttttggacaagagacgtggccgggaccctgagatggggggaaagccgagaaggaagaaccctcaggaaggcctgtacaatgaactgcagaaagataagatggcggaggcctacagtgagattgggatgaaaggcgagcgccggaggggcaaggggcacgatggcctttaccagggtctcagtacagccaccaaggacacctacgacgcccttcacatgcaggccctgccccctcgctaa

SEQ ID NO: 6 - DNA, 216 bp, Artificial Sequence
  Synthetic
actactaccaagccagtgctgcgaactccctcacctgtgcaccctaccgggacatctcagccccagagaccagaagattgtcggccccgtggctcagtgaaggggaccggattggacttcgcctgtgatatttacatctgggcacccttggccggaatctgcgtggcccttctgctgtccttgatcatcactctcatctgctaccacaggagccga

SEQ ID NO: 7 - DNA, 123 bp, Artificial Sequence
  Synthetic
aatagtagaaggaacagactccttcaagtgactaccatgaacatgactccccggaggcctgggctcactcgaaagccttaccagccctacgcccctgccagagactttgcagcgtaccgcccc

SEQ ID NO: 8 - DNA, 135 bp, Artificial Sequence
  Synthetic
aaatggatcaggaaaaaattcccccacatattcaagcaaccatttaagaagaccactggagcagctcaagaggaagatgcttgtagctgccgatgtccacaggaagaagaaggaggaggaggaggctatgagctg

SEQ ID NO: 9 - DNA, 339 bp, Artificial Sequence
  Synthetic
agagcaaaattcagcaggagtgcagagactgctgccaacctgcaggaccccaaccagctctacaatgagctcaatctagggcgaagagaggaatatgacgtcttggagaagaagcgggctcgcgatccagagatgggaggcaaacagcagaggaggaggaacccccaggaaggcgtatacaatgcactgcagaaagacaagatggcagaagcctacagtgagatcggcacaaaaggcgagaggcggagaggcaaggggcacgatggcctttaccagggtctcagcactgccaccaaggacacctatgatgccctgcatatgcagaccctggcccctcgc

SEQ ID NO: 10 - protein, 266 aa, Artificial Sequence
  Synthetic
MALPVTALLLPLALLLHAARPEVQLLESGGGLVQPGGSLRLSCAASGFTFSNAWMSWVRQAPGKGLEWVSYISSSGSTIYYADSVKGRFTISRDNSKNTLYLQMNSLRAEDTAVYYCAREGLWAFDKWGQGTLVTVSSGGGGSGGGGSGGGGSQSVLTQPPSASGTPGQRVTISCTGSSSNIGAGYVVHWYQQLPGTAPKLLIYDNNKRPSGVPDRFSGSKSGTSASLAISGLRSEDEADYYCAAFDDRLNGPVFGGGTKLTVLGQ

SEQ ID NO: 11 - protein, 83 aa, Artificial Sequence
  Synthetic
FVPVFLPAKPTTTPAPRPPTPAPTIASQPLSLRPEACRPAAGGAVHTRGLDFACDIYIWAPLAGTCGVLLLSLVITLYCNHRN

SEQ ID NO: 12 - protein, 41 aa, Artificial Sequence
  Synthetic
RSKRSRLLHSDYMNMTPRRPGPTRKHYQPYAPPRDFAAYRS

SEQ ID NO: 13 - protein, 47 aa, Artificial Sequence
  Synthetic
RFSVVKRGRKKLLYIFKQPFMRPVQTTQEEDGCSCRFPEEEEGGCEL

SEQ ID NO: 14 - protein, 112 aa, Artificial Sequence
  Synthetic
RVKFSRSADAPAYQQGQNQLYNELNLGRREEYDVLDKRRGRDPEMGGKPRRKNPQEGLYNELQKDKMAEAYSEIGMKGERRRGKGHDGLYQGLSTATKDTYDALHMQALPPR

SEQ ID NO: 15 - protein, 72 aa, Artificial Sequence
  Synthetic
TTTKPVLRTPSPVHPTGTSQPQRPEDCRPRGSVKGTGLDFACDIYIWAPLAGICVALLLSLIITLICYHRSR

SEQ ID NO: 16 - protein, 41 aa, Artificial Sequence
  Synthetic
NSRRNRLLQVTTMNMTPRRPGLTRKPYQPYAPARDFAAYRP

SEQ ID NO: 17 - protein, 45 aa, Artificial Sequence
  Synthetic
KWIRKKFPHIFKQPFKKTTGAAQEEDACSCRCPQEEEGGGGGYEL

SEQ ID NO: 18 - protein, 113 aa, Artificial Sequence
  Synthetic
RAKFSRSAETAANLQDPNQLYNELNLGRREEYDVLEKKRARDPEMGGKQQRRRNPQEGVYNALQKDKMAEAYSEIGTKGERRRGKGHDGLYQGLSTATKDTYDALHMQTLAPR

SEQ ID NO: 19 - DNA, 1642 bp, Homo sapiens
acatccaggggggacgccaagggagcaggacggagccatggaccccgccaggaaagcaggtgcccaggccatgatctggactgcaggctggctgctgctgctgctgcttcgcggaggagcgcaggccctggagtgctacagctgcgtgcagaaagcagatgacggatgctccccgaacaagatgaagacagtgaagtgcgcgccgggcgtggacgtctgcaccgaggccgtgggggcggtggagaccatccacggacaattctcgctggcagtgcggggttgcggttcgggactccccggcaagaatgaccgcggcctggatcttcacgggcttctggcgttcatccagctgcagcaatgcgctcaggatcgctgcaacgccaagctcaacctcacctcgcgggcgctcgacccggcaggtaatgagagtgcatacccgcccaacggcgtggagtgctacagctgtgtgggcctgagccgggaggcgtgccagggtacatcgccgccggtcgtgagctgctacaacgccagcgatcatgtctacaagggctgcttcgacggcaacgtcaccttgacggcagctaatgtgactgtgtccttgcctgtccggggctgtgtccaggatgaattctgcactcgggatggagtaacaggcccagggttcacgctcagtggctcctgttgccaggggtcccgctgtaactctgacctccgcaacaagacctacttctcccctcgaatcccaccccttgtccggctgccccctccagagcccacgactgtggcctcaaccacatctgtcaccacttctacctcggccccagtgagacccacatccaccaccaaacccatgccagcgccaaccagtcagactccgagacagggagtagaacacgaggcctcccgggatgaggagcccaggttgactggaggcgccgctggccaccaggaccgcagcaattcagggcagtatcctgcaaaaggggggccccagcagccccataataaaggctgtgtggctcccacagctggattggcagcccttctgttggccgtggctgctggtgtcctactgtgagcttctccacctggaaatttccctctcacctacttctctggccctgggtacccctcttctcatcacttcctgttcccaccactggactgggctggcccagcccctgtttttccaacattccccagtatccccagcttctgctgcgctggtttgcggctttgggaaataaaataccgttgtatatattctgccaggggtgttctagctttttgaggacagctcctgtatccttctcatccttgtctctccgcttgtcctcttgtgatgttaggacagagtgagagaagtcagctgtcacggggaaggtgagagagaggatgctaagcttcctactcactttctcctagccagcctggactttggagcgtggggtgggtgggacaatggctccccactctaagcactgcctcccctactccccgcatctttggggaatcggttccccatatgtcttccttactagactgtgagctcctcgagggcagggaccgtgccttatgtctgtgtgtgatcagtttctggcacataaatgcctcaataaagatttaattactttgtatagtg

SEQ ID NO: 20 - protein, 346 aa, Homo sapiens [sequence omitted]